European Patent Application EP 4 218 813 A2, published August 2, 2023. Title: HIGH CONCENTRATION ANTI-C5 ANTIBODY FORMULATIONS. Applicant: ALEXION PHARMACEUTICALS, INC. Application EP. The sequence listing filed with the application follows.

SEQUENCE LISTING (20 sequences)

SEQ ID NO: 1 - protein, 10 aa, synthetic construct
GYIFSNYWIQ

SEQ ID NO: 2 - protein, 17 aa, synthetic construct
EILPGSGSTEYTENFKD

SEQ ID NO: 3 - protein, 13 aa, synthetic construct
YFFGSSPNWYFDV

SEQ ID NO: 4 - protein, 11 aa, synthetic construct
GASENIYGALN

SEQ ID NO: 5 - protein, 7 aa, synthetic construct
GATNLAD

SEQ ID NO: 6 - protein, 9 aa, synthetic construct
QNVLNTPLT

SEQ ID NO: 7 - protein, 122 aa, synthetic construct [sequence omitted]

SEQ ID NO: 8 - protein, 107 aa, synthetic construct [sequence omitted]

SEQ ID NO: 9 - protein, 326 aa, synthetic construct
ASTKGPSVFPLAPCSRSTSESTAALGCLVKDYFPEPVTVSWNSGALTSGVHTFPAVLQSSGLYSLSSVVTVPSSNFGTQTYTCNVDHKPSNTKVDKTVERKCCVECPPCPAPPVAGPSVFLFPPKPKDTLMISRTPEVTCVVVDVSQEDPEVQFNWYVDGVEVHNAKTKPREEQFNSTYRVVSVLTVLHQDWLNGKEYKCKVSNKGLPSSIEKTISKAKGQPREPQVYTLPPSQEEMTKNQVSLTCLVKGFYPSDIAVEWESNGQPENNYKTTPPVLDSDGSFFLYSRLTVDKSRWQEGNVFSCSVMHEALHNHYTQKSLSLSLGK

SEQ ID NO: 10 - protein, 448 aa, synthetic construct
QVQLVQSGAEVKKPGASVKVSCKASGYIFSNYWIQWVRQAPGQGLEWMGEILPGSGSTEYTENFKDRVTMTRDTSTSTVYMELSSLRSEDTAVYYCARYFFGSSPNWYFDVWGQGTLVTVSSASTKGPSVFPLAPCSRSTSESTAALGCLVKDYFPEPVTVSWNSGALTSGVHTFPAVLQSSGLYSLSSVVTVPSSNFGTQTYTCNVDHKPSNTKVDKTVERKCCVECPPCPAPPVAGPSVFLFPPKPKDTLMISRTPEVTCVVVDVSQEDPEVQFNWYVDGVEVHNAKTKPREEQFNSTYRVVSVLTVLHQDWLNGKEYKCKVSNKGLPSSIEKTISKAKGQPREPQVYTLPPSQEEMTKNQVSLTCLVKGFYPSDIAVEWESNGQPENNYKTTPPVLDSDGSFFLYSRLTVDKSRWQEGNVFSCSVMHEALHNHYTQKSLSLSLGK

SEQ ID NO: 11 - protein, 214 aa, synthetic construct [sequence omitted]

SEQ ID NO: 12 - protein, 122 aa, synthetic construct [sequence omitted]

SEQ ID NO: 13 - protein, 326 aa, synthetic construct
ASTKGPSVFPLAPCSRSTSESTAALGCLVKDYFPEPVTVSWNSGALTSGVHTFPAVLQSSGLYSLSSVVTVPSSNFGTQTYTCNVDHKPSNTKVDKTVERKCCVECPPCPAPPVAGPSVFLFPPKPKDTLMISRTPEVTCVVVDVSQEDPEVQFNWYVDGVEVHNAKTKPREEQFNSTYRVVSVLTVLHQDWLNGKEYKCKVSNKGLPSSIEKTISKAKGQPREPQVYTLPPSQEEMTKNQVSLTCLVKGFYPSDIAVEWESNGQPENNYKTTPPVLDSDGSFFLYSRLTVDKSRWQEGNVFSCSVLHEALHSHYTQKSLSLSLGK

SEQ ID NO: 14 - protein, 448 aa, synthetic construct
QVQLVQSGAEVKKPGASVKVSCKASGHIFSNYWIQWVRQAPGQGLEWMGEILPGSGHTEYTENFKDRVTMTRDTSTSTVYMELSSLRSEDTAVYYCARYFFGSSPNWYFDVWGQGTLVTVSSASTKGPSVFPLAPCSRSTSESTAALGCLVKDYFPEPVTVSWNSGALTSGVHTFPAVLQSSGLYSLSSVVTVPSSNFGTQTYTCNVDHKPSNTKVDKTVERKCCVECPPCPAPPVAGPSVFLFPPKPKDTLMISRTPEVTCVVVDVSQEDPEVQFNWYVDGVEVHNAKTKPREEQFNSTYRVVSVLTVLHQDWLNGKEYKCKVSNKGLPSSIEKTISKAKGQPREPQVYTLPPSQEEMTKNQVSLTCLVKGFYPSDIAVEWESNGQPENNYKTTPPVLDSDGSFFLYSRLTVDKSRWQEGNVFSCSVLHEALHSHYTQKSLSLSLGK

SEQ ID NO: 15 - protein, 326 aa, synthetic construct
ASTKGPSVFPLAPCSRSTSESTAALGCLVKDYFPEPVTVSWNSGALTSGVHTFPAVLQSSGLYSLSSVVTVTSSNFGTQTYTCNVDHKPSNTKVDKTVERKCCVECPPCPAPPVAGPSVFLFPPKPKDTLYITREPEVTCVVVDVSHEDPEVQFNWYVDGMEVHNAKTKPREEQFNSTFRVVSVLTVVHQDWLNGKEYKCKVSNKGLPAPIEKTISKTKGQPREPQVYTLPPSREEMTKNQVSLTCLVKGFYPSDIAVEWESNGQPENNYKTTPPMLDSDGSFFLYSKLTVDKSRWQQGNVFSCSVMHEALHNHYTQKSLSLSPGK

SEQ ID NO: 16 - protein, 448 aa, synthetic construct
QVQLVQSGAEVKKPGASVKVSCKASGYIFSNYWIQWVRQAPGQGLEWMGEILPGSGSTEYTENFKDRVTMTRDTSTSTVYMELSSLRSEDTAVYYCARYFFGSSPNWYFDVWGQGTLVTVSSASTKGPSVFPLAPCSRSTSESTAALGCLVKDYFPEPVTVSWNSGALTSGVHTFPAVLQSSGLYSLSSVVTVTSSNFGTQTYTCNVDHKPSNTKVDKTVERKCCVECPPCPAPPVAGPSVFLFPPKPKDTLYITREPEVTCVVVDVSHEDPEVQFNWYVDGMEVHNAKTKPREEQFNSTFRVVSVLTVVHQDWLNGKEYKCKVSNKGLPAPIEKTISKTKGQPREPQVYTLPPSREEMTKNQVSLTCLVKGFYPSDIAVEWESNGQPENNYKTTPPMLDSDGSFFLYSKLTVDKSRWQQGNVFSCSVMHEALHNHYTQKSLSLSPGK

SEQ ID NO: 17 - protein, 11 aa, synthetic construct
GASENIYHALN

SEQ ID NO: 18 - protein, 17 aa, synthetic construct
EILPGSGHTEYTENFKD

SEQ ID NO: 19 - protein, 10 aa, synthetic construct
GHIFSNYWIQ

SEQ ID NO: 20 - protein, 448 aa, synthetic construct
QVQLVQSGAEVKKPGASVKVSCKASGHIFSNYWIQWVRQAPGQGLEWMGEILPGSGHTEYTENFKDRVTMTRDTSTSTVYMELSSLRSEDTAVYYCARYFFGSSPNWYFDVWGQGTLVTVSSASTKGPSVFPLAPCSRSTSESTAALGCLVKDYFPEPVTVSWNSGALTSGVHTFPAVLQSSGLYSLSSVVTVPSSNFGTQTYTCNVDHKPSNTKVDKTVERKCCVECPPCPAPPVAGPSVFLFPPKPKDTLMISRTPEVTCVVVDVSQEDPEVQFNWYVDGVEVHNAKTKPREEQFNSTYRVVSVLTVLHQDWLNGKEYKCKVSNKGLPSSIEKTISKAKGQPREPQVYTLPPSQEEMTKNQVSLTCLVKGFYPSDIAVEWESNGQPENNYKTTPPVLDSDGSFFLYSRLTVDKSRWQEGNVFSCSVMHEALHNHYTQKSLSLSLGK